European Patent Specification EP 2 790 708 B1, published October 23, 2024. Title: COMPOSITIONS AND METHODS FOR MODIFYING A PREDETERMINED TARGET NUCLEIC ACID SEQUENCE. Applicant: TargetGene Biotechnologies LTD. The sequence listing filed with the application follows.

SEQUENCE LISTING (217 sequences)

SEQ ID NO: 1 - DNA, 13 bp, Artificial sequence
  polynucleotide
cucuguaucuugu

SEQ ID NO: 2 - DNA, 25 bp, Artificial sequence
  polynucleotide
gtttacccgccaatatatcctgtca

SEQ ID NO: 3 - protein, 7 aa, Artificial sequence
  peptide
PKKKRKV

SEQ ID NO: 4 - protein, 25 aa, Artificial sequence
  Peptide
MLSLRQSIRFFKPATRTLCSSRYLL

SEQ ID NO: 5 - protein, 33 aa, Artificial sequence
  polypeptide
MLSALARPASAALRRSFSTSAQNNAKVAVLGAS

SEQ ID NO: 6 - protein, 23 aa, Artificial sequence
  polypeptide
MHSRSALLYRFLRPASRCFSSSS

SEQ ID NO: 7 - protein, 5 aa, Artificial sequence
  peptide
GGSGG

SEQ ID NO: 8 - protein, 12 aa, Artificial sequence
  peptide
NIHHVTWHMDFP

SEQ ID NO: 9 - protein, 7 aa, Artificial sequence
  peptide
PNSLIVP

SEQ ID NO: 10 - protein, 6 aa, Artificial sequence
  peptide
TGLDSP

SEQ ID NO: 11 - protein, 4 aa, Artificial sequence
  peptide
GSLE

SEQ ID NO: 12 - protein, 461 aa, Artificial sequence
  Artificial peptide
MPKKKRKVVKSELEEKKSELRHKLKYVPHEYIELIEIARNSTQDRILEMKVMEFFMKVYGYRGKHLGGSRKPDGAIYTVGSPIDYGVIVDTKAYSGGYNLPIGQADEMQRYVEENQTRNKHINPNEWWKVYPSSVTEFKFLFVSGHFKGNYKAQLTRLNHITNCNGAVLSVEELLIGGEMIKAGTLTLEEVRRKFNNGEINFGSLEGGSGGFDPEVQLQQSGPELVKPGASVRMSCKSSGYIFTDFYMNWVRQSHGKSLDYIGYISPYSGVTGYNQKFKGKATLTVDKSSSTAYMELRSLTSEDSAVYYCAGSSGNKWAMDYWGHGASVTVSSGGGGSGGGGSGGGGSDVVMTQTPLSLPVSLGDQASISCRSSQSLVHSNGNTYLNWYLQKAGQSPKLLIYKVSNRFSGVPDRFSGSGSGTDFTLKISRVEAEDLGIYFCSQTTHVPPTFGGGTKLEIKR

SEQ ID NO: 13 - DNA, 1386 bp, Artificial sequence
  Polynucleotide
atgcccaaaaagaaacgtaaagttgtgaaatcggaactcgaagagaagaaatccgagctcaggcataagttgaagtatgttccgcacgagtacattgaactaattgagatcgctcgtaactctacacaagaccgtattcttgaaatgaaggtgatggagtttttcatgaaggtttatggatatagagggaagcacttgggtggttctcgaaaacctgatggcgcaatctacacggttggctcgccaattgattatggggtgatagtggatactaaggcatactctggtggatacaatcttcctataggtcaagccgacgaaatgcagaggtatgttgaagaaaatcagacaagaaacaagcatatcaatcccaatgagtggtggaaggtttaccctagctctgtgaccgaattcaaattcttatttgtctccggtcactttaagggaaactataaggctcaattgacaagacttaatcatattacaaactgtaatggtgcagtgctcagtgtcgaagagttgcttataggtggggagatgattaaagccggaacgcttaccttggaagaagtacgtagaaaattcaataacggggagataaactttggaagcttagagggtggaagtggtggcttcgatccggaagtccagctccaacaaagtggacctgaactagttaagcctggcgcatccgttagaatgtcttgtaaatcaagtggatacatctttacagatttctacatgaactgggttaggcaatctcatgggaagtctcttgattacattggctatatctctccatattctggtgtaactgggtacaatcagaagtttaaaggtaaggctactttaactgtcgataaatcatcttctacagcgtatatggagttaagatcactgacatccgaagattcagctgtgtattactgtgctgggagttctgggaataagtgggcgatggactattggggccatggtgcttcggtcaccgtatcaagtggcggtggcggatccggtggtggtggctcgggtggtggcggaagtgacgttgtaatgacacaaaccccactgtctcttcctgtcagcctaggtgatcaggctagcatttcttgccgatcctcacaatctttagtgcactcgaatggaaacacttatcttaactggtacttgcagaaggcaggacagtcaccaaaactcttgatctataaagtttcaaacagattctcaggagttcctgacaggtttagcggaagcggatcgggaacagatttcacgctgaaaatctcacgcgttgaggctgaggatctcggtatttacttttgcagccaaactactcatgtgccaccgacttttgggggtggaacgaaattggagataaagaggtga

SEQ ID NO: 14 - protein, 9 aa, Artificial sequence
  peptide
GSLEGGSGG

SEQ ID NO: 15 - DNA, 1875 bp, Artificial sequence
  polynucleotide
gacaacatgtggagcacgacacacttgtctactccaaaaatatcaaagatacagtctcagaagaccaaagggcaattgagacttttcaacaaagggtaatatccggaaacctcctcggattccattgcccagctatctgtcactttattgtgaagatagtggaaaaggaaggtggctcctacaaatgccatcattgcgataaaggaaaggccatcgttgaagatgcctctgccgacagtggtcccaaagatggacccccacccacgaggagcatcgtggaaaaagaagacgttccaaccacgtcttcaaagcaagtggattgatgtgataacatggtggagcacgacacacttgtctactccaaaaatatcaaagatacagtctcagaagaccaaagggcaattgagacttttcaacaaagggtaatatccggaaacctcctcggattccattgcccagctatctgtcactttattgtgaagatagtggaaaaggaaggtggctcctacaaatgccatcattgcgataaaggaaaggccatcgttgaagatgcctctgccgacagtggtcccaaagatggacccccacccacgaggagcatcgtggaaaaagaagacgttccaaccacgtcttcaaagcaagtggattgatgtgatatctccactgacgtaagggatgacgcacaatcccactatccttcgcaagacccttcctctatataaggaagttcatttcatttggagaggacgtcgagagttctcaacacaacatatacaaaacaaacgaatctcaagcaatcaagcattctacttctattgcagcaatttaaatcatttcttttaaagcaaaagcaattttctgaaaattttcaccatttacgaacgatagccatggccgtcgacaactagtccagatctgtgtccaagggcgaggagctgttcaccggggtggtgcccatcctggtcgagctggacggcgacgtaaacggccacaagttcagcgtgtccggcgagggcgagggcgatgccacctacggcaagctgaccctgaagttcatctgcaccaccggcaagctgcccgtgccctggcccaccctcgtgaccaccctgacctacggcgtgcagtgcttcagccgctaccccgaccacatgaagcagcacgacttcttcaagtccgccatgcccgaaggctacgtccaggagcgcaccatcttcttcaaggacgacggcaactacaagacccgcgccgaggtgaagttcgagggcgacaccctggtgaaccgcatcgagctgaagggcatcgacttcaaggaggacggcaacatcctggggcacaagctggagtacaactacaacagccacaacgtctatatcatggccgacaagcagaagaacggcatcaaggtgaacttcaagatccgccacaacatcgaggacggcagcgtgcagctcgccgaccactaccagcagaacacccccatcggcgacggccccgtgctgctgcccgacaaccactacctgagcacccagtccgccctgagcaaagaccccaacgagaagcgcgatcacatggtcctgctggagttcgtgaccgccgccgggatcactctcggcatggacgagctgtacaagtccggactctaagcttgggtctagagtccgcaaaaatcaccagtctctctctacaaatctatctctctctatttttctccagaataatgtgtgagtagttcccagataagggaattagggttcttatagggtttcgctcatgtgttgagcatataagaaacccttagtatgtatttgtatttgtaaaatacttctatcaataaaatttctaattcctaaaaccaaaatccagtgacgcggccgc

SEQ ID NO: 16 - DNA, 712 bp, Artificial sequence
  polynucleotide
atggtgagcaagggcgaggaggataacatggccatcatcaaggagttcatgcccttcaaggtgcacatggagggctccgtgaacggccacgagttcgagatcgagggcgagggcgagggccgcccctacgagggcacccagaccgccaagctgaaggtgaccaagggtggccccctgcccttcgcctgggacatcctgtcccctcagttcatgtacggctccaaggcctacgtgaagcaccccgccgacatccccgactacttgaagctgtccttccccgagggcttcaagtgggagcgcgtgatgaacttcgaggacggcggcgtggtgaccgtgacccaggactcctccctgcaggacggcgagttcatctacaaggtgaagctgcgcggcaccaacttcccctccgacggccccgtaatgcagaagaagaccatgggctgggaggcctcctccgagcggatgtaccccgaggacggcgccctgaagggcgagatcaagcagaggctgaagctgaaggacggcggccactacgacgctgaggtcaagaccacctacaaggccaagaagcccgtgcagctgcccggcgcctacaacgtcaacatcaagttggacatcacctcccacaacgaggactacaccatcgtggaacagtacgaacgcgccgagggccgccactccaccggcggcatggacgagctgtacaagataa

SEQ ID NO: 17 - DNA, 21 bp, Artificial sequence
  polynucleotide
gtcgacaactagtccagatct

SEQ ID NO: 18 - DNA, 28 bp, Artificial sequence
  polynucleotide
  misc_feature (1)..(6): n is a, c, g, t or u
nnnnnngtgtccaagggcgaggagctgt

SEQ ID NO: 19 - DNA, 28 bp, Artificial sequence
  polynucleotide
  misc_feature (23)..(28): n is a, c, g, t or u
tttacgaacgatagccatggccnnnnnn

SEQ ID NO: 20 - DNA, 24 bp, Artificial sequence
  polynucleotide
  misc_feature (1)..(2): n is a, c, g, t or u
nngtccaagggcgaggagctgttc

SEQ ID NO: 21 - DNA, 24 bp, Artificial sequence
  polynucleotide
  misc_feature (23)..(24): n is a, c, g, t or u
atttacgaacgatagccatggcnn

SEQ ID NO: 22 - DNA, 27 bp, Artificial sequence
  polynucleotide
  misc_feature (22)..(27): n is a, c, g, t or u
cagctcctcgcccttggagacnnnnnn

SEQ ID NO: 23 - DNA, 27 bp, Artificial sequence
  polynucleotide
  misc_feature (1)..(6): n is a, c, g, t or u
nnnnnnggccatggctatcgttcgtaa

SEQ ID NO: 24 - DNA, 24 bp, Artificial sequence
  polynucleotide
  misc_feature (23)..(24): n is a, c, g, t or u
gaacagctcctcgcccttggacnn

SEQ ID NO: 25 - DNA, 24 bp, Artificial sequence
  polynucleotide
  misc_feature (1)..(2): n is a, c, g, t or u
nngccatggctatcgttcgtaaat

SEQ ID NO: 26 - DNA, 21 bp, Artificial sequence
  polynucleotide
gactctaagcttgggtctaga

SEQ ID NO: 27 - DNA, 24 bp, Artificial sequence
  polynucleotide
  misc_feature (1)..(2): n is a, c, g, or t
nntccgcaaaaatcaccagtctct

SEQ ID NO: 28 - DNA, 24 bp, Artificial sequence
  polynucleotide
  misc_feature (23)..(24): n is a, c, g, or t
gcatggacgagctgtacaagtcnn

SEQ ID NO: 29 - DNA, 24 bp, Artificial sequence
  polynucleotide
  misc_feature (23)..(24): n is a, c, g, or t
agagactggtgatttttgcggann

SEQ ID NO: 30 - DNA, 24 bp, Artificial sequence
  polynucleotide
  misc_feature (1)..(2): n is a, c, g, or t
nngacttgtacagctcgtccatgc

SEQ ID NO: 31 - DNA, 22 bp, Artificial sequence
  polynucleotide
ctatccttcgcaagacccttcc

SEQ ID NO: 32 - DNA, 22 bp, Artificial sequence
  polynucleotide
ttatcttgtacagctcgtccat

SEQ ID NO: 33 - DNA, 22 bp, Artificial sequence
  polynucleotide
ccctataagaaccctaattccc

SEQ ID NO: 34 - DNA, 20 bp, Artificial sequence
  polynucleotide
atggtgagcaagggcgagga

SEQ ID NO: 35 - DNA, 21 bp, Artificial sequence
  polynucleotide
ttctcaagtcatgagcaactc

SEQ ID NO: 36 - DNA, 28 bp, Artificial sequence
  polynucleotide
  misc_feature (1)..(6): n is a, c, g, or t
nnnnnnctgtggggccatatcccagaac

SEQ ID NO: 37 - DNA, 28 bp, Artificial sequence
  polynucleotide
  misc_feature (23)..(28): n is a, c, g, or t
gcgggcaccgagttgtattgtannnnnn

SEQ ID NO: 38 - DNA, 28 bp, Artificial sequence
  polynucleotide
  misc_feature (23)..(28): n is a, c, g, or t
gttctgggatatggccccacagnnnnnn

SEQ ID NO: 39 - DNA, 28 bp, Artificial sequence
  polynucleotide
  misc_feature (1)..(6): n is a, c, g, or t
nnnnnntacaatacaactcggtgcccgc

SEQ ID NO: 40 - DNA, 23 bp, Artificial sequence
  polynucleotide
  misc_feature (1)..(2): n is a, c, g, or t
nngtggggccatatcccagaact

SEQ ID NO: 41 - DNA, 24 bp, Artificial sequence
  polynucleotide
  misc_feature (23)..(24): n is a, c, g, or t
agcgggcaccgagttgtattgtnn

SEQ ID NO: 42 - DNA, 24 bp, Artificial sequence
  polynucleotide
  misc_feature (1)..(2): n is a, c, g, or t
nnacaatacaactcggtgcccgct

SEQ ID NO: 43 - DNA, 23 bp, Artificial sequence
  polynucleotide
  misc_feature (22)..(23): n is a, c, g, or t
agttctgggatatggccccacnn

SEQ ID NO: 44 - DNA, 22 bp, Artificial sequence
  polynucleotide
gagctagatagcagatgcagat

SEQ ID NO: 45 - DNA, 22 bp, Artificial sequence
  polynucleotide
ctccagaaaatccctagaaaca

SEQ ID NO: 46 - DNA, 1988 bp, Artificial sequence
  polynucleotide
ggtgtctgacagcagaagatcctcgatggagatggatggggttctgcaagccgcggatgccaaggactgggtttacaagggggaaggcgccgcgaatctcatcctcagctacaccggctcgtcgccctccatggtaagcgctgagtaggttcttactgagcgtgcacgcatcgatcacttgactttaggggctcaatgtgtgattcacgggtgccgcggcgccattcgagctccagatccagtaccgctcgagcaagtgataaaacatggagcagggacgatcacgtggtcacttgaaaattacgtgaggtccggggcgacgatgtacggcgccggcgaactctcaaacactcacacaaccaaaaccgcttcgtgttcgtctttgttccaagcgactgtgtgagtgtttgagagttcgccagcgccgtacatcgtcgccccggatctgacaaattaagctttcgttgcttttccatgattgtgcattttgtgagcatgcactgaatactatgatggatatgtttggaggaagcattattccaatttgatgataagggtgttatttacacttgttttcagcttggcaaggtactgcggctcaagaagattctaaaaaacaagatgagcaagggcgaggagctgttcaccggggtggtgcccatcctggtcgagctggacggcgacgtaaacggccacaagttcagcgtgtccggcgagggcgagggcgatgccacctacggcaagctgaccctgaagttcatctgcaccaccggcaagctgcccgtgccctggcccaccctcgtgaccaccctgacctacggcgtgcagtgcttcagccgctaccccgaccacatgaagcagcacgacttcttcaagtccgccatgcccgaaggctacgtccaggagcgcaccatcttcttcaaggacgacggcaactacaagacccgcgccgaggtgaagttcgagggcgacaccctggtgaaccgcatcgagctgaagggcatcgacttcaaggaggacggcaacatcctggggcacaagctggagtacaactacaacagccacaacgtctatatcatggccgacaagcagaagaacggcatcaaggtgaacttcaagatccgccacaacatcgaggacggcagcgtgcagctcgccgaccactaccagcagaacacccccatcggcgacggccccgtgctgctgcccgacaaccactacctgagcacccagtccgccctgagcaaagaccccaacgagaagcgcgatcacatggtcctgctggagttcgtgaccgccgccgggatcactctcggcatggacgagctgtacaagtaactcaagcctatgcagtgcatgttatgagccaacacctgggtgccaatcatgtcgatggtggggtatggttcagattcagttcatttatgtcctgttattgtgattttgattggtaacatattgacaacctcgacacttgggatcagattcagttcacttatggaagaaattggagaattgttataatttatctataatcacccctactgaaatagaaataacatggcatcaatgtgcatgctattggattttgacacgaatatgctttattctatcatatgttggtaattccagcaggcagcaggcactactctttggatccacgtgacttgacaaagaaatcatgccatctttccacaatgcaggtccgtgtacgtgtttctagggattttctggagcttgtcgaaaagaatgttcttagcagccgtcctgctgggagagtaaatgcaagttcaattgataacactgctgatgccgctcttctaatagcagaccactctttattttctggtacgtactctatccctcttcttaccataatctgaatcttgttaaggtttaaaatatatgattgattaagtaaaatccagagctctattcatatctcatgcactgatgttttgatgaaacacttgtagcaagacggttgc

SEQ ID NO: 47 - DNA, 2987 bp, Artificial sequence
  polynucleotide
ggtgtctgacagcagaagatcctcgatggagatggatggggttctgcaagccgcggatgccaaggactgggtttacaagggggaaggcgccgcgaatctcatcctcagctacaccggctcgtcgccctccatggtaagcgctgagtaggttcttactgagcgtgcacgcatcgatcacttgactttaggggctcaatgtgtgattcacgggtgccgcggcgccattcgagctccagatccagtaccgctcgagcaagtgataaaacatggagcagggacgatcacgtggtcacttgaaaattacgtgaggtccggggcgacgatgtacggcgccggcgaactctcaaacactcacacaaccaaaaccgcttcgtgttcgtctttgttccaagcgactgtgtgagtgtttgagagttcgccagcgccgtacatcgtcgccccggatctgacaaattaagctttcgttgcttttccatgattgtgcattttgtgagcatgcactgaatactatgatggatatgtttggaggaagcattattccaatttgatgataagggtgttatttacacttgttttcagcttggcaaggtactgcggctcaagaagattctaaaaaacaagtaaatagtataaccggtcaacatgtggagcacgacacacttgtctactccaaaaatatcaaagatacagtctcagaagaccaaagggcaattgagacttttcaacaaagggtaatatccggaaacctcctcggattccattgcccagctatctgtcactttattgtgaagatagtggaaaaggaaggtggctcctacaaatgccatcattgcgataaaggaaaggccatcgttgaagatgcctctgccgacagtggtcccaaagatggacccccacccacgaggagcatcgtggaaaaagaagacgttccaaccacgtcttcaaagcaagtggattgatgtgataacatggtggagcacgacacacttgtctactccaaaaatatcaaagatacagtctcagaagaccaaagggcaattgagacttttcaacaaagggtaatatccggaaacctcctcggattccattgcccagctatctgtcactttattgtgaagatagtggaaaaggaaggtggctcctacaaatgccatcattgcgataaaggaaaggccatcgttgaagatgcctctgccgacagtggtcccaaagatggacccccacccacgaggagcatcgtggaaaaagaagacgttccaaccacgtcttcaaagcaagtggattgatgtgatatctccactgacgtaagggatgacgcacaatcccactatccttcgcaagacccttcctctatataaggaagttcatttcatttggagaggacgtcgagagttctcaacacaacatatacaaaacaaacgaatctcaagcaatcaagcattctacttctattgcagcaatttaaatcatttcttttaaagcaaaagcaattttctgaaaattttcaccatttacgaacgatagcatgagcccagaacgacgcccggccgacatccgccgtgccaccgaggcggacatgccggcggtctgcaccatcgtcaaccactacatcgagacaagcacggtcaacttccgtaccgagccgcaggaaccgcaggagtggacggacgacctcgtccgtctgcgggagcgctatccctggctcgtcgccgaggtggacggcgaggtcgccggcatcgcctacgcgggcccctggaaggcacgcaacgcctacgactggacggccgagtcgaccgtgtacgtctccccccgccaccagcggacgggactgggctccacgctctacacccacctgctgaagtccctggaggcacagggcttcaagagcgtggtcgctgtcatcgggctgcccaacgacccgagcgtgcgcatgcacgaggcgctcggatatgccccccgcggcatgctgcgggcggccggcttcaagcacgggaactggcatgacgtgggtttctggcagctggacttcagcctgccggtaccgccccgtccggtcctgcccgtcaccgagatctgatcccgatcgttcaaacatttggcaataaagtttcttaagattgaatcctgttgccggtcttgcgatgattatcatataatttctgttgaattacgttaagcatgtaataattaacatgtaatgcatgacgttatttatgagatgggtttttatgattagagtcccgcaattatacatttaatacgcgatagaaaacaaaatatagcgcgcaaactaggataaattatcgcgcgcggtgtcatctatgttactagatcgggctcaagcctatgcagtgcatgttatgagccaacacctgggtgccaatcatgtcgatggtggggtatggttcagattcagttcatttatgtcctgttattgtgattttgattggtaacatattgacaacctcgacacttgggatcagattcagttcacttatggaagaaattggagaattgttataatttatctataatcacccctactgaaatagaaataacatggcatcaatgtgcatgctattggattttgacacgaatatgctttattctatcatatgttggtaattccagcaggcagcaggcactactctttggatccacgtgacttgacaaagaaatcatgccatctttccacaatgcaggtccgtgtacgtgtttctagggattttctggagcttgtcgaaaagaatgttcttagcagccgtcctgctgggagagtaaatgcaagttcaattgataacactgctgatgccgctcttctaatagcagaccactctttattttctggtacgtactctatccctcttcttaccataatctgaatcttgttaaggtttaaaatatatgattgattaagtaaaatccagagctctattcatatctcatgcactgatgttttgatgaaacacttgtagcaagacggttgc

SEQ ID NO: 48 - DNA, 1672 bp, Artificial sequence
  polynucleotide
atggtcatttcttctggttcaagcatgacatgaacaggcaataaataagttgagattttgatcacagtaactgatacttgaatcgaatcatttagattttttttttttttagtttacttgtttagtaaatatgttgtctatgtttgtcacaaaaacgtggctcagttcttgtatatatggagacaaaaaaatccattaaaagattgttgacattctcggaaatttagtgccaactgttattgcgagaacttactatagttttcctttggcgaaaagctaataatcttaaatcttgattttgtcctcttttctctgagttagattttcttaaattccacttccgacctattaagaaatgggcttttgcaaagaagatccgcttcactgagcccgtatctcgaagaggataatacaacaacaaagcaaaacggcacgtagttttaattgtaaccaaggattgcatttcggtcttgtttcaacaaacgaaacttcctgaaatgccaagaaaaatctggtcatttcaccacagtgatcattgtgtatgtgttctaaagactccaagcgaaggttttagaaaaaggagcattttctattctattcaagaaactcgaagaacattctctcttcatcctctaacttccctataaatatgtcctttgctaatcagatcaaatcagcaggaaaatcaagaaccaaaagtctcccgaaaagcaacgaacaatggatcctgatgatgttgttgattcttctaaatcttttgtgatggaaaacttttcttcgtaccacgggactaaacctggttatgtagattccattcaaaaaggtatacaaaagccaaaatctggtacacaaggaaattatgacgatgattggaaagggttttatagtaccgacaataaatacgacgctgcgggatactctgtagataatgaaaacccgctctctggaaaagctggaggcgtggtcaaagtgacgtatccaggactgacgaaggttctcgcactaaaagtggataatgccgaaactattaagaaagagttaggtttaagtctcactgaaccgttgatggagcaagtcggaacggaagagtttatcaaaaggttcggtgatggtgcttcgcgtgtagtgctcagccttcccttcgctgaggggagttctagcgttgaatatattaataactgggaacaggcgaaagcgttaagcgtagaacttgagattaattttgaaacccgtggaaaacgtggccaagatgcgatgtatgagtatatggctcaagcctgtgcaggaaatcgtgtcaggcgatctctttgtgaaggaaccttacttctgtggtgtgacataattggacaaactacctacagagatttaaagctctaaggatcccccgggctgcaggaattcgatccgctagcatcgttcaaacatttggcaataaagtttcttaagattgaatcctgttgccggtcttgcgatgattatcatataatttctgttgaattacgttaagcatgtaataattaacatgtaatgcatgacgttatttatgagatgggtttttatgattagagtcccgcaattatacatttaatacgcgatagaaaacaaaatatagcgcgcaaactaggataaattatcgcgcgcggtgtcatctatgttactagatcgctagcgg

SEQ ID NO: 49 - protein, 462 aa, Artificial sequence
  polypeptide
MPKKKRKVVKSELEEKKSELRHKLKYVPHEYIELIEIARNSTQDRILEMKVMEFFMKVYGYRGKHLGGSRKPDGAIYTVGSPIDYGVIVDTKAYSGGYNLPIGQADEMQRYVEENQTRNKHINPNEWWKVYPSSVTEFKFLFVSGHFKGNYKAQLTRLNHITNCNGAVLSVEELLIGGEMIKAGTLTLEEVRRKFNNGEINFGGSGGSDVVMTQTPLSLPVSLGDQASISCRSSQSLVHSNGNTYLRWYLQKPGQSPKVLIYKVSNRFSGVPDRFSGSGSGTDFTLKISRVEAEDLGVYFCSQSTHVPWTFGGGTKLEIKSSADDAKKDAAKKDDAKKDDAKKDGGVKLDETGGGLVQPGRPMKLSCVASGFTFSDYWMNWVRQSPEKGLEWVAQIRNKPYNYETYYSDSVKGRFTISRDDSKSSVYLQMNNLRVEDMGIYYCTGSYYGMDYWGQGTSVTVS

SEQ ID NO: 50 - DNA, 1389 bp, Artificial sequence
  polynucleotide
atgccgaaaaagaagaggaaggtggtgaagagcgaactggaggagaaaaagtccgagctccgccacaagctgaagtacgtcccgcacgagtacatcgaactgatcgagattgccaggaattccacccaggaccgcatcctcgaaatgaaggtcatggaattcttcatgaaggtgtacggctaccgcgggaaacacctcggcggcagcaggaagccagatggcgcgatctatacggtcgggtccccgatcgactatggggtgatcgtcgacaccaaagcgtacagcggcggctacaacctcccaattggccaggcggacgagatgcagaggtatgtggaggagaaccagacccgcaataagcacatcaacccgaacgagtggtggaaggtgtacccaagctccgtgaccgagttcaagttcctcttcgtgtccgggcacttcaagggcaattacaaggcccagctgacgcgcctcaaccatatcacgaattgcaatggcgccgtcctgtccgtcgaagagctgctcatcggcggggagatgatcaaggcgggcacgctgacgctggaggaagtacgtaggaaattcaacaacggggaaatcaatttcgggggatccgggggcagcgatgtggtgatgacgcagaccccactgtccctgccagtgtccctaggcgaccaagcgagcatctcctgtcgcagcagccagtccctcgtgcactccaacggcaacacgtatctccgctggtatctccagaagccggggcagtccccgaaagtgctgatctacaaggtctccaaccgcttctccggcgtcccggataggtttagcggcagcgggtccggcaccgactttaccctgaaaatctccagggtggaggccgaggatctcggggtctacttttgcagccagagcacgcacgtcccatggacctttgggggcggcacgaaactggagattaaaagcagcgctgacgatgccaagaaggacgcggcgaaaaaggacgacgccaagaaagacgacgcgaaaaaagacggcggcgtcaagctcgatgaaaccggcggcgggctcgtgcaaccaggccgcccgatgaagcttagctgcgtggccagcgggttcaccttcagcgactactggatgaactgggtccgccaatccccggaaaagggcctggagtgggtggcccagatcaggaacaagccatataactatgagacgtactactccgatagcgtgaaagggcgcttcaccatctccagggacgacagcaagtcctccgtgtacctccagatgaacaacctacgcgtggaggatatgggcatctactactgcaccgggagctactacggcatggactactggggccagggcacgtccgtcaccgtgtcctga

SEQ ID NO: 51 - DNA, 21 bp, Artificial sequence
  polynucleotide
gtcctgctaagcctttgaaag

SEQ ID NO: 52 - DNA, 28 bp, Artificial sequence
  polynucleotide
  misc_feature (23)..(28): n is a, c, g, or t
gcatccttccgtagtgctcctcnnnnnn

SEQ ID NO: 53 - DNA, 28 bp, Artificial sequence
  polynucleotide
  misc_feature (1)..(6): n is a, c, g, or t
nnnnnnttgtaattgctggtgctggtat

SEQ ID NO: 54 - DNA, 28 bp, Artificial sequence
  polynucleotide
  misc_feature (1)..(6): n is a, c, g, or t
nnnnnngaggagcactacggaaggatgc

SEQ ID NO: 55 - DNA, 24 bp, Artificial sequence
  polynucleotide
  misc_feature (23)..(24): n is a, c, g, or t
tgcatccttccgtagtgctcctnn

SEQ ID NO: 56 - DNA, 24 bp, Artificial sequence
  polynucleotide
  misc_feature (1)..(2): n is a, c, g, or t
nngtaattgctggtgctggtatgt

SEQ ID NO: 57 - DNA, 24 bp, Artificial sequence
  polynucleotide
  misc_feature (1)..(2): n is a, c, g, or t
nnaggagcactacggaaggatgca

SEQ ID NO: 58 - DNA, 24 bp, Artificial sequence
  polynucleotide
  misc_feature (23)..(24): n is a, c, g, or t
acataccagcaccagcaattacnn

SEQ ID NO: 59 - DNA, 1865 bp, Artificial sequence
  polynucleotide
aaattacgttgagatgcatggtctctctctactcaattaaccaaataaggaaaagaatcatatggtcatcaattcgtaaatcaaaattttaatttgtgtggtatttaatccatctacatgtttcgtaagcaacaaaagagcttggtctgaaaaccaaacaagaccatatgggcactcgaatactccattttgttatcggctacttccactagcctcctccttcgctgcgtctcctgtttctctacttcacgattactcgctaggtaaaagataagatactaaacaactactatagcccctttaattcaagtccgtttttttttgttcttcttcttttcaattatgtgttaaagatacaaacttttgtctgatttgcttccaccggtttcacctaagatactcaattttcttactttttgtgtgttttgtaattctaattcttttatagcttcaatttttagattcattgaagcagttgtgagttaagttggagaaaatggttgtgtttgggaatgtttctgcggcgaatttgccttatcaaaacgggtttttggaggcactttcatctggaggttgtgaactaatgggacatagctttagggttcccacttctcaagcgcttaagacaagaacaaggaggaggagtactgctggtcctttgatggtgagcaagggcgaggaggataacatggccatcatcaaggagttcatgcccttcaaggtgcacatggagggctccgtgaacggccacgagttcgagatcgagggcgagggcgagggccgcccctacgagggcacccagaccgccaagctgaaggtgaccaagggtggccccctgcccttcgcctgggacatcctgtcccctcagttcatgtacggctccaaggcctacgtgaagcaccccgccgacatccccgactacttgaagctgtccttccccgagggcttcaagtgggagcgcgtgatgaacttcgaggacggcggcgtggtgaccgtgacccaggactcctccctgcaggacggcgagttcatctacaaggtgaagctgcgcggcaccaacttcccctccgacggccccgtaatgcagaagaagaccatgggctgggaggcctcctccgagcggatgtaccccgaggacggcgccctgaagggcgagatcaagcagaggctgaagctgaaggacggcggccactacgacgctgaggtcaagaccacctacaaggccaagaagcccgtgcagctgcccggcgcctacaacgtcaacatcaagttggacatcacctcccacaacgaggactacaccatcgtggaacagtacgaacgcgccgagggccgccactccaccggcggcatggacgagctgtacaagtaaggtatgtctacaacttcatttcttactgctttgtttgggatctgatggaattaatgttcatgtgatgaagttcttttggctctcaaataattgcaggattggctggattgtcaactgcaaagtacctggctgatgcaggccacaaacctctgttgcttgaagcaagagatgttcttggtggaaaggtactttgattggtctcactttccgaattacttattgttgtttgcatttctcattcttatatgatttgctgattcccaaaggctgtaccaattatgtttgtgagactacaaggtataactagtgtttagagtgttacagctcctaggtacccaatgtatctgtcctgtttgttgtattagtcttgtactgcccaatttgttttttattatgttctaatgtcttcagtcttgtgctacacaccgcacaaccctttccagtttctaggcttaatgtgaatcaaatatagagtagtttactggaagatatc

SEQ ID NO: 60 - DNA, 23 bp, Artificial sequence
  polynucleotide
tggttgtgtttgggaatgtttct

SEQ ID NO: 61 - DNA, 26 bp, Artificial sequence
  polynucleotide
tatccaaaagatatcttccagtaaac

SEQ ID NO: 62 - RNA, 20 nt, Artificial sequence
  polynucleoitde
uucaccucuaaccgggugag

SEQ ID NO: 63 - protein, 18 aa, Artificial sequence
  polypeptide
GTAKSRYKARRAELIAER

SEQ ID NO: 64 - DNA, 21 bp, Artificial sequence
  polynucleotide
ggtcaagtgccacgtaggatg

SEQ ID NO: 65 - DNA, 21 bp, Artificial sequence
  polynucleotide
ggtcaagtggcgcgcaggatg

SEQ ID NO: 66 - protein, 194 aa, Artificial polypeptide
  polypeptide
VKSELEEKKSELRHKLKYVPHEYIELIEIARNSTQDRILEMKVMEFFMKVYGYRGKHLGGSRKPDGAIYTVGSPIDYGVIVDTKAYSGGYNLPIGQADEMQRYVEENQTRNKHINPNEWWKVYPSSVTEFKFLFVSGHFKGNYKAQLTRLNHITNCNGAVLSVEELLIGGEMIKAGTLTLEEVRRKFNNGEINF

SEQ ID NO: 67 - protein, 8 aa, Artificial sequence
  peptide
MPKKKRKV

SEQ ID NO: 68 - protein, 225 aa, Artificial sequence
  polypeptide
MGTAKSRYKARRAELIAERGGSGGVKSELEEKKSELRHKLKYVPHEYIELIEIARNSTQDRILEMKVMEFFMKVYGYRGKHLGGSRKPDGAIYTVGSPIDYGVIVDTKAYSGGYNLPIGQADEMQRYVEENQTRNKHINPNEWWKVYPSSVTEFKFLFVSGHFKGNYKAQLTRLNHITNCNGAVLSVEELLIGGEMIKAGTLTLEEVRRKFNNGEINFPKKKRKV

SEQ ID NO: 69 - DNA, 678 bp, Artificial sequence
  polypeptide
atggggacggccaagtccaggtacaaggcgcgcagggccgaactgattgcggagaggggcggatccggcggcgtcaaatccgagctcgaagagaagaagagcgagctgaggcacaagctgaagtacgtcccgcacgagtacatcgaactcatcgagatcgccaggaactccacccaggaccgcatcctggagatgaaggtgatggagttcttcatgaaggtgtacggctaccgtggcaaacatctggggggctccaggaaaccggatggggccatctacaccgtggggagcccgatcgactacggcgtgatcgtggacaccaaagcgtactccggcggctacaacctcccgattggccaggccgatgaaatgcagcgctacgtggaggagaaccagacgcgcaataagcacatcaacccgaacgagtggtggaaggtgtacccgtcctccgtgaccgagttcaagttcctgttcgtgagcggccacttcaaggggaactacaaggcccagctgacccgcctgaaccacatcaccaactgcaatggggcggtgctctccgtggaggaactcctgatcggcggcgagatgatcaaggccggcaccctgaccctggaagaggtacgtagaaagttcaacaacggcgagatcaacttcccgaagaagaagcgcaaggtgtga

SEQ ID NO: 70 - RNA, 43 nt, Artificial sequence
  polynucleotide
  misc_feature (21)..(21): n is a, c, g, or u
uucaccucuaaccgggugagngguacugaugcuuuucaggaaa

SEQ ID NO: 71 - RNA, 43 nt, Artificial sequence
  polynucleotide
  misc_feature (23)..(23): n is a, c, g, or u
auagcguccccauuguugcuaunuucaccucuaaccgggugag

SEQ ID NO: 72 - RNA, 43 nt, Artificial sequence
  polynucleotide
  misc_feature (23)..(23): n is a, c, g, or u
uuuccugaaaagcaucaguaccnuucaccucuaaccgggugag

SEQ ID NO: 73 - RNA, 42 nt, Artificial sequence
  polynucleotide
  misc_feature (20)..(20): n is a, c, g, or u
ucaccucuaaccgggugagnauagcaacaauggggacgcuau

SEQ ID NO: 74 - protein, 8 aa, Artificial sequence
  peptide
GGSGGESK

SEQ ID NO: 75 - protein, 229 aa, Artificial sequence
  polypeptide
MPKKKRKVVKSELEEKKSELRHKLKYVPHEYIELIEIARNSTQDRILEMKVMEFFMKVYGYRGKHLGGSRKPDGAIYTVGSPIDYGVIVDTKAYSGGYNLPIGQADEMQRYVEENQTRNKHINPNEWWKVYPSSVTEFKFLFVSGHFKGNYKAQLTRLNHITNCNGAVLSVEELLIGGEMIKAGTLTLEEVRRKFNNGEINFGGSGGESKGTAKSRYKARRAELIAERR

SEQ ID NO: 76 - DNA, 690 bp, Artificial sequence
  polypeptide
atgccaaagaagaagagaaaggttgttaagtctgaacttgaagaaaagaagtctgaacttagacataagcttaagtatgttccacatgaatatattgaacttattgaaattgctagaaattctactcaagatagaattcttgaaatgaaggttatggaattttttatgaaggtttatggatatagaggaaagcatcttggaggatctagaaagccagatggagctatttatactgttggatctccaattgattatggagttattgttgatactaaggcttattctggaggatataatcttccaattggacaagctgatgaaatgcaaagatatgttgaagaaaatcaaactagaaataagcatattaatccaaatgaatggtggaaggtttatccatcttctgttactgaatttaagtttctttttgtttctggacattttaagggaaattataaggctcaacttactagacttaatcatattactaattgtaatggagctgttctttctgttgaagaacttcttattggaggagaaatgattaaggctggaactcttactcttgaagaagttagaagaaagtttaataatggagaaattaattttggaggatctggaggagaatctaagggaactgctaagtctagatataaggctagaagagctgaacttattgctgaaagaagataa

SEQ ID NO: 77 - RNA, 42 nt, Artificial sequence
  polynucleotide
uucaccucuaaccgggugaguacugaugcuuuucaggaaacu

SEQ ID NO: 78 - RNA, 42 nt, Artificial sequence
  polynucleotide
gauagcguccccauuguugcuauucaccucuaaccgggugag

SEQ ID NO: 79 - RNA, 42 nt, Artificial
  polynucleotide
aguuuccugaaaagcaucaguauucaccucuaaccgggugag

SEQ ID NO: 80 - RNA, 42 nt, Artificial sequence
  polynucleotide
uucaccucuaaccgggugaguagcaacaauggggacgcuauc

SEQ ID NO: 81 - RNA, 43 nt, Artificial sequence
  polynucleotide
  misc_feature (21)..(21): n is a, c, g, or u
uucaccucuaaccgggugagnucgguacugaugcuuuucagga

SEQ ID NO: 82 - RNA, 43 nt, Artificial sequence
  polynucleotide
  misc_feature (23)..(23): n is a, c, g, or u
gcguccccauuguugcuauaacnuucaccucuaaccgggugag

SEQ ID NO: 83 - RNA, 43 nt, Artificial sequence
  polynucleotide
  misc_feature (23)..(23): n is a, c, g, or u
uccugaaaagcaucaguaccganuucaccucuaaccgggugag

SEQ ID NO: 84 - RNA, 43 nt, Artificial sequence
  polynucleotide
  misc_feature (21)..(21): n is a, c, g, or u
uucaccucuaaccgggugagnguuauagcaacaauggggacgc

SEQ ID NO: 85 - DNA, 1995 bp, Artificial sequence
  polynucleotide
atggcggcggctgcggcggctccatctccctctttctccaaaaccctatcgtcctcctcctccaaatcctccaccctcctccctagatccaccttccctttcccccaccacccccacaaaaccaccccaccacccctccacctcacccccacccacattcacagccaacgccgtcgtttcaccatctccaatgtcatttccactacccaaaaagtttccgagacccaaaaagccgaaactttcgtttcccgttttgcccctgacgaacccagaaagggttccgacgttctcgtggaggccctcgaaagagaaggggttacggacgtttttgcgtacccaggcggcgcttccatggagattcaccaagctttgacgcgctcaagcatcatccgcaacgtgctaccacgtcacgagcagggtggtgtcttcgccgctgagggttacgcacgcgccaccggcttccccggcgtttgcattgccacctccggccctggcgccaccaatctcgtcagtggcctcgcggacgccctactggatagcgtccccattgttgctataaccggtcaagtgccacgtaggatgatcggtactgatgcttttcaggaaactccgattgttgaggtaactagatcgattaccaagcataattatctcgttatggacgtagaggatattcctagggttgtacgtgaggcttttttccttgcgagatcgggccggcctggccctgttttgattgatgtacctaaggatattcagcaacaattggtgatacctgactgggatcagccaatgaggttgcctggttacatgtctaggttacctaaattgcccaatgagatgcttttagaacaaattgttaggcttatttctgagtcaaagaagcctgttttgtatgtggggggtgggtgttcgcaatcgagtgaggagttgagacgattcgtggagctcaccggtatccccgtggcaagtactttgatgggtcttggagcttttccaactggggatgagctttccctttcaatgttgggtatgcatggtactgtttatgctaattatgctgtggacagtagtgatttattgctcgcatttggggtgaggtttgatgatagagttactggaaagttagaagcttttgctagccgagcgaaaattgttcacattgatattgattcagctgagattggaaagaacaagcagcctcatgtttccatttgtgcggatatcaagttggcgttacagggtttgaattcgatattggagagtaaggaaggtaaactgaagttggatttttctgcttggaggcaggagttgacggtgcagaaagtgaagtacccgttgaattttaaaacttttggtgatgctattcctccgcaatatgctatccaggttctagatgagttaactaatgggagtgctattataagtaccggtgttgggcagcaccagatgtgggctgctcaatattataagtacagaaagccacgccaatggttgacatctggtggattaggagcgatgggatttggtttgcccgctgctattggtgcggctgttggaagacctgatgaagttgtggttgacattgatggtgatggcagtttcatcatgaatgtgcaggagctagcaactattaaggtggagaatctcccagttaagattatgttactgaataatcaacacttgggaatggtggttcaatgggaggatcggttctataaggctaacagagcacacacatacctggggaatccttctaatgaggcggagatctttcctaatatgttgaaatttgcagaggcttgtggcgtacctgctgcgagagtgacacacagggatgatcttagagcggctattcaaaagatgttagacactcctgggccatacttgttggatgtgattgtacctcatcaggaacatgttctacctatgattcccagtggcggggctttcaaagatgtgatcacagagggtgacgggagaagttcctattga

SEQ ID NO: 86 - DNA, 1995 bp, Artificial sequence
  polynucleotide
atggcggcggctgcggcggctccatctccctctttctccaaaaccctatcgtcctcctcctccaaatcctccaccctcctccctagatccaccttccctttcccccaccacccccacaaaaccaccccaccacccctccacctcacccccacccacattcacagccaacgccgtcgtttcaccatctccaatgtcatttccactacccaaaaagtttccgagacccaaaaagccgaaactttcgtttcccgttttgcccctgacgaacccagaaagggttccgacgttctcgtggaggccctcgaaagagaaggggttacggacgtttttgcgtacccaggcggcgcttccatggagattcaccaagctttgacgcgctcaagcatcatccgcaacgtgctaccacgtcacgagcagggtggtgtcttcgccgctgagggttacgcacgcgccaccggcttccccggcgtttgcattgccacctccggccctggcgccaccaatctcgtcagtggcctcgcggacgccctactggatagcgtcccaatagtagccataactggtcaagtggcgcgcaggatgatcggtaccgatgcttttcaggaaactccgattgttgaggtaactagatcgattaccaagcataattatctcgttatggacgtagaggatattcctagggttgtacgtgaggcttttttccttgcgagatcgggccggcctggccctgttttgattgatgtacctaaggatattcagcaacaattggtgatacctgactgggatcagccaatgaggttgcctggttacatgtctaggttacctaaattgcccaatgagatgcttttagaacaaattgttaggcttatttctgagtcaaagaagcctgttttgtatgtggggggtgggtgttcgcaatcgagtgaggagttgagacgattcgtggagctcaccggtatccccgtggcaagtactttgatgggtcttggagcttttccaactggggatgagctttccctttcaatgttgggtatgcatggtactgtttatgctaattatgctgtggacagtagtgatttattgctcgcatttggggtgaggtttgatgatagagttactggaaagttagaagcttttgctagccgagcgaaaattgttcacattgatattgattcagctgagattggaaagaacaagcagcctcatgtttccatttgtgcggatatcaagttggcgttacagggtttgaattcgatattggagagtaaggaaggtaaactgaagttggatttttctgcttggaggcaggagttgacggtgcagaaagtgaagtacccgttgaattttaaaacttttggtgatgctattcctccgcaatatgctatccaggttctagatgagttaactaatgggagtgctattataagtaccggtgttgggcagcaccagatgtgggctgctcaatattataagtacagaaagccacgccaatggttgacatctggtggattaggagcgatgggatttggtttgcccgctgctattggtgcggctgttggaagacctgatgaagttgtggttgacattgatggtgatggcagtttcatcatgaatgtgcaggagctagcaactattaaggtggagaatctcccagttaagattatgttactgaataatcaacacttgggaatggtggttcaatgggaggatcggttctataaggctaacagagcacacacatacctggggaatccttctaatgaggcggagatctttcctaatatgttgaaatttgcagaggcttgtggcgtacctgctgcgagagtgacacacagggatgatcttagagcggctattcaaaagatgttagacactcctgggccatacttgttggatgtgattgtacctcatcaggaacatgttctacctatgattcccagtggcggggctttcaaagatgtgatcacagagggtgacgggagaagttcctattga

SEQ ID NO: 87 - protein, 286 aa, Artificial sequence
  polypeptide
PAEKRKPIRVLSLFDGIATGLLVLKDLGIQVDRYIASEVCEDSITVGMVRHQGKIMYVGDVRSVTQKHIQEWGPFDLVIGGSPCNDLSIVNPARKGLYEGTGALFFEFYRLLHDARPKEGDDRPFFWLFENVVAMGVSDKRDISRFLESNPVMIDAKEVSAAHRARYFWGNLPGMNRPLASTVNDKLELQECLEHGRIAKFSKVRTITTRSNSIKQGKDQHFPVFMNEKEDILWCTEMERVFGFPVHYTDVSNMSRLARQRLLGRSWSVPVIRHLFAPLKEYFACV

SEQ ID NO: 88 - protein, 557 aa, Artificial sequence
  polypeptide
MPKKKRKVDVVMTQTPLSLPVSLGDQASISCRSSQSLVHSNGNTYLRWYLQKPGQSPKVLIYKVSNRFSGVPDRFSGSGSGTDFTLKISRVEAEDLGVYFCSQSTHVPWTFGGGTKLEIKSSADDAKKDAAKKDDAKKDDAKKDGGVKLDETGGGLVQPGRPMKLSCVASGFTFSDYWMNWVRQSPEKGLEWVAQIRNKPYNYETYYSDSVKGRFTISRDDSKSSVYLQMNNLRVEDMGIYYCTGSYYGMDYWGQGTSVTVSGSLEGGSGGPAEKRKPIRVLSLFDGIATGLLVLKDLGIQVDRYIASEVCEDSITVGMVRHQGKIMYVGDVRSVTQKHIQEWGPFDLVIGGSPCNDLSIVNPARKGLYEGTGALFFEFYRLLHDARPKEGDDRPFFWLFENVVAMGVSDKRDISRFLESNPVMIDAKEVSAAHRARYFWGNLPGMNRPLASTVNDKLELQECLEHGRIAKFSKVRTITTRSNSIKQGKDQHFPVFMNEKEDILWCTEMERVFGFPVHYTDVSNMSRLARQRLLGRSWSVPVIRHLFAPLKEYFACV

SEQ ID NO: 89 - DNA, 1674 bp, Artificial sequence
  polynucleotide
atgcctaagaagaagagaaaggttgatgttgttatgactcaaactcctctttctcttcctgtttctcttggagatcaagcttctatttcttgtagatcttctcaatctcttgttcattctaatggaaatacttatcttagatggtatcttcaaaagcctggacaatctcctaaggttcttatttataaggtttctaatagattttctggagttcctgatagattttctggatctggatctggaactgattttactcttaagatttctagagttgaagctgaagatcttggagtttatttttgttctcaatctactcatgttccttggacttttggaggaggaactaagcttgaaattaagtcttctgctgatgatgctaagaaggatgctgctaagaaggatgatgctaagaaggatgatgctaagaaggatggaggagttaagcttgatgaaactggaggaggacttgttcaacctggaagacctatgaagctttcttgtgttgcttctggatttactttttctgattattggatgaattgggttagacaatctcctgaaaagggacttgaatgggttgctcaaattagaaataagccttataattatgaaacttattattctgattctgttaagggaagatttactatttctagagatgattctaagtcttctgtttatcttcaaatgaataatcttagagttgaagatatgggaatttattattgtactggatcttattatggaatggattattggggacaaggaacttctgttactgtttctggatctcttgaaggaggatctggaggacctgctgaaaagagaaagcctattagagttctttctctttttgatggaattgctactggacttcttgttcttaaggatcttggaattcaagttgatagatatattgcttctgaagtttgtgaagattctattactgttggaatggttagacatcaaggaaagattatgtatgttggagatgttagatctgttactcaaaagcatattcaagaatggggaccttttgatcttgttattggaggatctccttgtaatgatctttctattgttaatcctgctagaaagggactttatgaaggaactggagctcttttttttgaattttatagacttcttcatgatgctagacctaaggaaggagatgatagaccttttttttggctttttgaaaatgttgttgctatgggagtttctgataagagagatatttctagatttcttgaatctaatcctgttatgattgatgctaaggaagtttctgctgctcatagagctagatatttttggggaaatcttcctggaatgaatagacctcttgcttctactgttaatgataagcttgaacttcaagaatgtcttgaacatggaagaattgctaagttttctaaggttagaactattactactagatctaattctattaagcaaggaaaggatcaacattttcctgtttttatgaatgaaaaggaagatattctttggtgtactgaaatggaaagagtttttggatttcctgttcattatactgatgtttctaatatgtctagacttgctagacaaagacttcttggaagatcttggtctgttcctgttattagacatctttttgctcctcttaaggaatattttgcttgtgtttaa

SEQ ID NO: 90 - DNA, 1896 bp, Artificial sequence
  polynucleotide
accggtcaacatgtggagcacgacacacttgtctactccaaaaatatcaaagatacagtctcagaagaccaaagggcaattgagacttttcaacaaagggtaatatccggaaacctcctcggattccattgcccagctatctgtcactttattgtgaagatagtggaaaaggaaggtggctcctacaaatgccatcattgcgataaaggaaaggccatcgttgaagatgcctctgccgacagtggtcccaaagatggacccccacccacgaggagcatcgtggaaaaagaagacgttccaaccacgtcttcaaagcaagtggattgatgtgataacatggtggagcacgacacacttgtctactccaaaaatatcaaagatacagtctcagaagaccaaagggcaattgagacttttcaacaaagggtaatatccggaaacctcctcggattccattgcccagctatctgtcactttattgtgaagatagtggaaaaggaaggtggctcctacaaatgccatcattgcgataaaggaaaggccatcgttgaagatgcctctgccgacagtggtcccaaagatggacccccacccacgaggagcatcgtggaaaaagaagacgttccaaccacgtcttcaaagcaagtggattgatgtgatatctccactgacgtaagggatgacgcacaatcccactatccttcgcaagacccttcctctatataaggaagttcatttcatttggagaggacgtcgagagttctcaacacaacatatacaaaacaaacgaatctcaagcaatcaagcattctacttctattgcagcaatttaaatcatttcttttaaagcaaaagcaattttctgaaaattttcaccatttacgaacgatagagatctcgagctcaagcttcgaattctgcagtcgacggtaccgcgggcccgggatcctgatggtgagcaagggcgaggaggataacatggccatcatcaaggagttcatgcccttcaaggtgcacatggagggctccgtgaacggccacgagttcgagatcgagggcgagggcgagggccgcccctacgagggcacccagaccgccaagctgaaggtgaccaagggtggccccctgcccttcgcctgggacatcctgtcccctcagttcatgtacggctccaaggcctacgtgaagcaccccgccgacatccccgactacttgaagctgtccttccccgagggcttcaagtgggagcgcgtgatgaacttcgaggacggcggcgtggtgaccgtgacccaggactcctccctgcaggacggcgagttcatctacaaggtgaagctgcgcggcaccaacttcccctccgacggccccgtaatgcagaagaagaccatgggctgggaggcctcctccgagcggatgtaccccgaggacggcgccctgaagggcgagatcaagcagaggctgaagctgaaggacggcggccactacgacgctgaggtcaagaccacctacaaggccaagaagcccgtgcagctgcccggcgcctacaacgtcaacatcaagttggacatcacctcccacaacgaggactacaccatcgtggaacagtacgaacgcgccgagggccgccactccaccggcggcatggacgagctgtacaagagatccacctgatctagagtccgcaaaaatcaccagtctctctctacaaatctatctctctctatttttctccagaataatgtgtgagtagttcccagataagggaattagggttcttatagggtttcgctcatgtgttgagcatataagaaacccttagtatgtatttgtatttgtaaaatacttctatcaataaaatttctaattcctaaaaccaaaatccagtgacgcggccgc

SEQ ID NO: 91 - DNA, 28 bp, Artificial sequence
  polynucleotide
  misc_feature (23)..(28): n is a, c, g, or t
tcgagctcaagcttcgaattctnnnnnn

SEQ ID NO: 92 - DNA, 28 bp, Artificial sequence
  polynucleotide
  misc_feature (1)..(6): n is a, c, g, or t
nnnnnngatggtgagcaagggcgaggag

SEQ ID NO: 93 - protein, 17 aa, Artificial sequence
  peptide
SGPRPRGTRGKGRRIRR

SEQ ID NO: 94 - RNA, 31 nt, Artificial sequence
  polynucleotide
uucagcucguguagcucauuagcuccgagcu

SEQ ID NO: 95 - DNA, 31 bp, Artificial sequence
  polynucleotide
ttccatacagtcagtatcaattctggaagaa

SEQ ID NO: 96 - DNA, 22 bp, Artificial sequence
  polypeptide
atcaattctggaagaatttcca

SEQ ID NO: 97 - DNA, 22 bp, Artificial sequence
  polynucleotide
tcattacacctgcagctctcat

SEQ ID NO: 98 - DNA, 53 bp, Artificial sequence
  polynucleotide
uucagcucguguagcucauuagcuccgagcuaucaauucuggaagaauuucca

SEQ ID NO: 99 - DNA, 53 bp, Artificial sequence
  polynucleotide
ucauuacaccugcagcucucauuucagcucguguagcucauuagcuccgagcu

SEQ ID NO: 100 - RNA, 55 nt, Artificial sequence
  polynucleotide
  misc_feature (32)..(33): n is a, c, g, or u
uucagcucguguagcucauuagcuccgagcunnguaucaauucuggaagaauuuc

SEQ ID NO: 101 - DNA, 56 bp, Artificial sequence
  polynucleotide
  misc_feature (24)..(25): n is a, c, g, t or u
caaaaagaaggucuucauuacacnnuucagcucguguagcucauuagcuccgagcu

SEQ ID NO: 102 - DNA, 32 bp, Artificial sequence
  polynucleotide
tttccatacagtcagtatcaattctggaagaa

SEQ ID NO: 103 - DNA, 31 bp, Artificial sequence
  polynucleotide
cagggtggaacaagatggattatcaagtgtc

SEQ ID NO: 104 - DNA, 53 bp, Artificial sequence
  polynucleotide
uucagcucguguagcucauuagcuccgagcuaagtccaatctatgacatcaat

SEQ ID NO: 105 - DNA, 53 bp, Artificial sequence
  polynucleotide
aagatcactttttatttatgcauucagcucguguagcucauuagcuccgagcu

SEQ ID NO: 106 - DNA, 55 bp, Artificial sequence
  polynucleotide
  misc_feature (32)..(33): n is a, c, g, t or u
uucagcucguguagcucauuagcuccgagcunnucaaguccaaucuaugacauca

SEQ ID NO: 107 - DNA, 55 bp, Artificial sequence
  polynucleotide
  misc_feature (23)..(24): n is a, c, g, t or u
gaucacuuuuuauuuaugcacannuucagcucguguagcucauuagcuccgagcu

SEQ ID NO: 108 - DNA, 31 bp, Artificial sequence
  polynucleotide
atatctgtgggcttgtgacacggactcaagt

SEQ ID NO: 109 - DNA, 53 bp, Artificial sequence
  polynucleotide
uucagcucguguagcucauuagcuccgagcugggctggtgacccagtcagagt

SEQ ID NO: 110 - DNA, 53 bp, Artificial sequence
  polynucleotide
ccgatccactggggagcaggaauucagcucguguagcucauuagcuccgagcu

SEQ ID NO: 111 - DNA, 55 bp, Artificial sequence
  polynucleotide
  misc_feature (32)..(33): n is a, c, g, t or u
uucagcucguguagcucauuagcuccgagcunnugggcuggugacccagucagag

SEQ ID NO: 112 - DNA, 55 bp, Artificial sequence
  polynucleotide
  misc_feature (23)..(24): n is a, c, g, t or u
auccacuggggagcaggaaauannuucagcucguguagcucauuagcuccgagcu

SEQ ID NO: 113 - protein, 7 aa, Artificial sequence
  peptide
GSGGSGP

SEQ ID NO: 114 - protein, 223 aa, Artificial sequence
  polypeptide
MPKKKRKVVKSELEEKKSELRHKLKYVPHEYIELIEIARNSTQDRILEMKVMEFFMKVYGYRGKHLGGSRKPDGAIYTVGSPIDYGVIVDTKAYSGGYNLPIGQADEMQRYVEENQTRNKHINPNEWWKVYPSSVTEFKFLFVSGHFKGNYKAQLTRLNHITNCNGAVLSVEELLIGGEMIKAGTLTLEEVRRKFNNGEINFGSGGSGPRPRGTRGKGRRIRR

SEQ ID NO: 115 - DNA, 672 bp, Artificial sequence
  polypeptide
atgcccaagaagaagagaaaggtggtgaagagcgagctggaggagaagaagagcgagctgagacacaagctgaagtacgtgccccacgagtacatcgagctgatcgagatcgccagaaacagcacccaggacagaatcctggagatgaaggtgatggagttcttcatgaaggtgtacggctacagaggcaagcacctgggcggcagcagaaagcccgacggcgccatctacaccgtgggcagccccatcgactacggcgtgatcgtggacaccaaggcctacagcggcggctacaacctgcccatcggccaggccgacgagatgcagagatacgtggaggagaaccagaccagaaacaagcacatcaaccccaacgagtggtggaaggtgtaccccagcagcgtgaccgagttcaagttcctgttcgtgagcggccacttcaagggcaactacaaggcccagctgaccagactgaaccacatcaccaactgcaacggcgccgtgctgagcgtggaggagctgctgatcggcggcgagatgatcaaggccggcaccctgaccctggaggaggtgagaagaaagttcaacaacggcgagatcaacttcggcagcggcggcagcggccccagacccagaggcaccagaggcaagggcagaagaatcagaagataa

SEQ ID NO: 116 - protein, 7 aa, Artificial sequence
  peptide
GGSGGGP

SEQ ID NO: 117 - DNA, 31 bp, Artificial sequence
  polynucleotide
uucagcucguguagcucauuagcuccgagcu

SEQ ID NO: 118 - DNA, 31 bp, Artificial sequence
  polynucleotide
gcaaaacaattatttggttatgccattttgg

SEQ ID NO: 119 - DNA, 53 bp, Artificial sequence
  polynucleotide
uucagcucguguagcucauuagcuccgagcucaaugauggauuucgcgccacg

SEQ ID NO: 120 - DNA, 53 bp, Artificial sequence
  polynucleotide
uuagcuucgguuagagcaaagcuucagcucguguagcucauuagcuccgagcu

SEQ ID NO: 121 - DNA, 53 bp, Artificial sequence
  polynucleotide
uucagcucguguagcucauuagcuccgagcugccaaugauggauuucgcgcca

SEQ ID NO: 122 - DNA, 53 bp, Artificial sequence
  polynucleotide
agcuucgguuagagcaaagcccuucagcucguguagcucauuagcuccgagcu

SEQ ID NO: 123 - DNA, 22 bp, Artificial sequence
  polynucleotide
atgttagaaggtgcaaaatcaa

SEQ ID NO: 124 - DNA, 22 bp, Artificial sequence
  polynucleotide
ctaacggacttggaatacgaat

SEQ ID NO: 125 - DNA, 2833 bp, Artificial sequence
  polynucleotide
tgctgtaccatacagtctttccgcttaaagaattatattctctctagctacttcacagtgtcctttcctttcgcgtactcctctgtctttttcctatcttctctcttctattaccgagacccgtacatacaaagatctaggtagctcatctccttctaagaagtcagatctccttcctatattctataaagaataagagcccttcttaacttcactctttaattgtaaagagaggcctcatttaggagcgctgttttcatccaactatcaatctcgtaagagaataaagcgtggaaaagaaaggttttgattcgctttataaagaagaaagctttttccggttctaacaggctaattaaattagaaacgcgtctgttcacgtcaggtccgaagggatgtggttgcttttccttttttgcgtcgagattgggttggtgttcagtgtaccgcttgtctagcctatgctttgcatgaacatctcaatgtccaagataaaaagaacgaggggaagaatcgacgaggccagtgttctcgaagagaaaatcgtgatggaaaaagcgtgaggagaattcgaaagtcgatatgttagaaggtgcaaaatcaatgggtgcaggagctgctacaatcgcttcagcgggagctgctatcggtattggaaacgtccttagttcctcgattcattccgtgttaggtatacaaataacagacttacatcacgatgtctttttcttcgttattctgattttggttttcgtatcatggatcttgggtcgcgctttatggcatttccactataaaaaaaatccaatcccgcaaaggattgttcatggaactactatcgagattcttcggaccttatttcttagtatcatccctatgttcattgctataccatcatttgccctgtatgggtattcggactataacagttccgatgaacagtcactcacttttgacagttatacgattccagaagatcatccagaattgggtcaatcacgtttattagaagtcgacaatagagtggttgtaccagcaaacagttctctccgttttattgtaacatctgcggctgtaccttccttaggtgtcaaaggtgatgctgtgccttccttaggtgtcaaaggtgatgctgtgccttccttaggtgtcaaaggtgatgctgtgcctgggcctgggcgggtttttcagacttggacccgagcttttgagcgtttgggcctgttgacggttgcccattgcgccggcaccggaacatcaagctcgggctcggtagtcagtcttccacaggacgaaatatgggccgcccttgagggcgatccccaggcccttccggaagacggccaatttcacgccgtcgcccctgaggggaatccccaggcccttccggaagacgggcaatttcacgccgtcccccctgaggggaatccccaggcccttccggaagacgggcaatttcaggccgtcgcccctgaggggaatccccaggcccttccggaagacgggcaatttcacgccatcgcctttgaccctcttatagcaacacggcaagacgcgtggaatacgctacttgtcttgttgcggcgcagcaccaaaattggcctaaggccaattttgttactaaagcaggggaagatcttggtatagaggaggtcgactttaaaagcgaacgaaaaacaattgcaaaagcagattgatttttggcaacgtgaatttaggttttggaagtaaaataagttttatttgataaaaattgctaattcagtataattaatatttacgaggtgacataacgtatgaaaaaatcagaggattattcctcctaaatataaaaatttaaaatttaggaggaagttatatatgacttttaatattattgaattagaaaattgggatagaaaagaatattttgaacactattttaatcagcaaactacttatagcattactaaagaaattgatattactttgtttaaagatatgataaaaaagaaaggatatgaaatttatccctctttaatttatgcaattatggaagttgtaaataaaaataaagtgtttagaacaggaattaatagtgagaataaattaggttattgggataagttaaatcctttgtatacagtttttaataagcaaactgaaaaatttactaacatttggactgaatctgataaaaacttcatttctttttataataattataaaaatgacttgcttgaatataaagataaagaagaaatgtttcctaaaaaaccgatacctgaaaacaccataccgatttcaatgattccttggattgattttagttcatttaatttaaatattggtaacaatagcagctttttattgcctattattacgataggtaaattttatagtgagaataataaaatttatataccagttgctctgcaacttcatcattctgtatgtgatggttaccatgcttcactatttatgaatgaatttcaagatataattcatagggtagatgattggatttagtttttagattttgaaagtgaatttaattttatacacgtaagtgatcaggagggaagctaatgcatcgtttgccccaatgatggcctttttgatctcattcgtattccaagtccgttagtcatcgtttacggtgggtgggtaagcaggaggggatccctgtggttagattagagtaactggccgagaaggttagcgaggttccagctatggtgaagtgaaagatctttcacttcactatagtgggaaagaagacaggtgggagcgagcggagcgagagcaaagcaagctctagtggtgggttgtcttcgcggtcccatttcatcga

SEQ ID NO: 126 - DNA, 31 bp, Artificial sequence
  polynucleotide
agacttacatcacgatgtctttttcttcgtt

SEQ ID NO: 127 - DNA, 53 bp, Artificial sequence
  polynucleotide
uucagcucguguagcucauuagcuccgagcuguuauuuguauaccuaacacgg

SEQ ID NO: 128 - DNA, 53 bp, Artificial sequence
  polynucleotide
auacgaaaaccaaaaucagaauuucagcucguguagcucauuagcuccgagcu

SEQ ID NO: 129 - DNA, 53 bp, Artificial sequence
  polynucleotide
uucagcucguguagcucauuagcuccgagcucuguuauuuguauaccuaacac

SEQ ID NO: 130 - DNA, 53 bp, Artificial sequence
  polynucleotide
acgaaaaccaaaaucagaauaauucagcucguguagcucauuagcuccgagcu

SEQ ID NO: 131 - DNA, 2852 bp, Artificial sequence
  polynucleotide
tgctgtaccatacagtctttccgcttaaagaattatattctctctagctacttcacagtgtcctttcctttcgcgtactcctctgtctttttcctatcttctctcttctattaccgagacccgtacatacaaagatctaggtagctcatctccttctaagaagtcagatctccttcctatattctataaagaataagagcccttcttaacttcactctttaattgtaaagagaggcctcatttaggagcgctgttttcatccaactatcaatctcgtaagagaataaagcgtggaaaagaaaggttttgattcgctttataaagaagaaagctttttccggttctaacaggctaattaaattagaaacgcgtctgttcacgtcaggtccgaagggatgtggttgcttttccttttttgcgtcgagattgggttggtgttcagtgtaccgcttgtctagcctatgctttgcatgaacatctcaatgtccaagataaaaagaacgaggggaagaatcgacgaggccagtgttctcgaagagaaaatcgtgatggaaaaagcgtgaggagaattcgaaagtcgatatgttagaaggtgcaaaatcaatgggtgcaggagctgctacaaatgcttcagcgggagctgctatcggtattggaaacgtccttagttcctcgattcattccgtggcgcgaaatccatcattggcaaaacaattatttggttatgccattttgggctttgctctaaccgaagctaatgcatcgtttgccccaatgatggcctttttgatctcattcgtattccaagtccgttagaggaggtcgactttaaaagcgaacgaaaaacaattgcaaaagcagattgatttttggcaacgtgaatttaggttttggaagtaaaataagttttatttgataaaaattgctaattcagtataattaatatttacgaggtgacataacgtatgaaaaaatcagaggattattcctcctaaatataaaaatttaaaatttaggaggaagttatatatgacttttaatattattgaattagaaaattgggatagaaaagaatattttgaacactattttaatcagcaaactacttatagcattactaaagaaattgatattactttgtttaaagatatgataaaaaagaaaggatatgaaatttatccctctttaatttatgcaattatggaagttgtaaataaaaataaagtgtttagaacaggaattaatagtgagaataaattaggttattgggataagttaaatcctttgtatacagtttttaataagcaaactgaaaaatttactaacatttggactgaatctgataaaaacttcatttctttttataataattataaaaatgacttgcttgaatataaagataaagaagaaatgtttcctaaaaaaccgatacctgaaaacaccataccgatttcaatgattccttggattgattttagttcatttaatttaaatattggtaacaatagcagctttttattgcctattattacgataggtaaattttatagtgagaataataaaatttatataccagttgctctgcaacttcatcattctgtatgtgatggttaccatgcttcactatttatgaatgaatttcaagatataattcatagggtagatgattggatttagtttttagattttgaaagtgaatttaattttatacacgtaagtgatcaggaggaaaaaatccaatcccgcaaaggattgttcatggaactactatcgagattcttcggaccttatttcttagtatcatccctatgttcattgctataccatcatttgccctgtatgggtattcggactataacagttccgatgaacagtcactcacttttgacagttatacgattccagaagatcatccagaattgggtcaatcacgtttattagaagtcgacaatagagtggttgtaccagcaaacagttctctccgttttattgtaacatctgcggctgtaccttccttaggtgtcaaaggtgatgctgtgccttccttaggtgtcaaaggtgatgctgtgccttccttaggtgtcaaaggtgatgctgtgcctgggcctgggcgggtttttcagacttggacccgagcttttgagcgtttgggcctgttgacggttgcccattgcgccggcaccggaacatcaagctcgggctcggtagtcagtcttccacaggacgaaatatgggccgcccttgagggcgatccccaggcccttccggaagacggccaatttcacgccgtcgcccctgaggggaatccccaggcccttccggaagacgggcaatttcacgccgtcccccctgaggggaatccccaggcccttccggaagacgggcaatttcaggccgtcgcccctgaggggaatccccaggcccttccggaagacgggcaatttcacgccatcgcctttgaccctcttatagcaacacggcaagacgcgtggaatacgctacttgtcttgttgcggcgcagcaccaaaattggcctaaggccaattttgttactaaagcaggggaagatcttggtataggaagctaatgcatcgtttgccccaatgatggcctttttgatctcattcgtattccaagtccgttagtcatcgtttacggtgggtgggtaagcaggaggggatccctgtggttagattagagtaactggccgagaaggttagcgaggttccagctatggtgaagtgaaagatctttcacttcactatagtgggaaagaagacaggtgggagcgagcggagcgagagcaaagcaagctctagtggtgggttgtcttcgcggtcccatttcatcga

SEQ ID NO: 132 - protein, 399 aa, Artificial sequence
  polypeptide
MDKAELIPEPPKKKRKVELGTAANFNQSGNIADSSLSFTFTNSSNGPNLITTQTNSQALSQPIASSNVHDNFMNNEITASKIDDGNNSKPLSPGWTDQTAYNAFGITTGMFNTTTMDDVYNYLFDDEDTPPNPKKEGSLEGGSGGDVVMTQTPLSLPVSLGDQASISCRSSQSLVHSNGNTYLRWYLQKPGQSPKVLIYKVSNRFSGVPDRFSGSGSGTDFTLKISRVEAEDLGVYFCSQSTHVPWTFGGGTKLEIKSSADDAKKDAAKKDDAKKDDAKKDGGVKLDETGGGLVQPGRPMKLSCVASGFTFSDYWMNWVRQSPEKGLEWVAQIRNKPYNYETYYSDSVKGRFTISRDDSKSSVYLQMNNLRVEDMGIYYCTGSYYGMDYWGQGTSVTVS

SEQ ID NO: 133 - DNA, 21 bp, Artificial sequence
  polynucleotide
gggcatctggaccctcctacc

SEQ ID NO: 134 - DNA, 28 bp, Artificial sequence
  polynucleotide
  misc_feature (23)..(28): n is a, c, g, t or u
aggattgctcaacaaccatgctnnnnnn

SEQ ID NO: 135 - DNA, 28 bp, Artificial sequence
  polynucleotide
  misc_feature (1)..(6): n is a, c, g, t or u
nnnnnntctggtgagccctctcctgccc

SEQ ID NO: 136 - DNA, 24 bp, Artificial sequence
  polynucleotide
  misc_feature (23)..(24): n is a, c, g, t or u
ggaggattgctcaacaaccatgnn

SEQ ID NO: 137 - DNA, 24 bp, Artificial sequence
  polynucleotide
  misc_feature (1)..(2): n is a, c, g, t or u
nnctggtgagccctctcctgcccg

SEQ ID NO: 138 - DNA, 21 bp, Artificial sequence
  polynucleotide
tacgtctgttgctagattatc

SEQ ID NO: 139 - DNA, 28 bp, Artificial sequence
  polynucleotide
  misc_feature (23)..(28): n is a, c, g, t or u
atgcttttattttacaggttctnnnnnn

SEQ ID NO: 140 - DNA, 28 bp, Artificial sequence
  polynucleotide
  misc_feature (1)..(6): n is a, c, g, t or u
nnnnnngtccaaaagtgttaatgcccaa

SEQ ID NO: 141 - DNA, 24 bp, Artificial sequence
  polynucleotide
  misc_feature (23)..(24): n is a, c, g, t or u
tcatgcttttattttacaggttnn

SEQ ID NO: 142 - DNA, 24 bp, Artificial sequence
  polynucleotide
  misc_feature (1)..(2): n is a, c, g, t or u
nntccaaaagtgttaatgcccaag

SEQ ID NO: 143 - DNA, 21 bp, Artificial sequence
  polynucleotide
cagttgagactcagaacttgg

SEQ ID NO: 144 - DNA, 29 bp, Artificial sequence
  polynucleotide
  misc_feature (24)..(29): n is a, c, g, t or u
ggaattgaggaagactgttactannnnnn

SEQ ID NO: 145 - DNA, 34 bp, Artificial sequence
  polynucleotide
  misc_feature (1)..(6): n is a, c, g, t or u
nnnnnnaaggcctgcatcatgatggccaattctc

SEQ ID NO: 146 - DNA, 24 bp, Artificial sequence
  polynucleotide
  misc_feature (23)..(24): n is a, c, g, t or u
ggaattgaggaagactgttactnn

SEQ ID NO: 147 - DNA, 24 bp, Artificial sequence
  polynucleotide
  misc_feature (1)..(2): n is a, c, g, t or u
nnggcctgcatcatgatggccaat

SEQ ID NO: 148 - DNA, 18 bp, Artificial sequence
  polynucleotide
catgcttttattttacag

SEQ ID NO: 149 - DNA, 20 bp, Artificial sequence
  polynucleotide
ctgtgactttcactgtaatc

SEQ ID NO: 150 - DNA, 21 bp, Artificial sequence
  polynucleotide
caattgtgaattcacatagaa

SEQ ID NO: 151 - DNA, 28 bp, Artificial sequence
  polynucleotide
  misc_feature (23)..(28): n is a, c, g, t or u
ggtgtcatattatacaatatttnnnnnn

SEQ ID NO: 152 - DNA, 28 bp, Artificial sequence
  polynucleotide
  misc_feature (1)..(6): n is a, c, g, t or u
nnnnnnaacattaaattataatgtttga

SEQ ID NO: 153 - DNA, 24 bp, Artificial sequence
  polynucleotide
  misc_feature (23)..(24): n is a, c, g, t or u
ttggtgtcatattatacaatatnn

SEQ ID NO: 154 - DNA, 24 bp, Artificial sequence
  polynucleotide
  misc_feature (1)..(2): n is a, c, g, t or u
nnacattaaattataatgtttgac

SEQ ID NO: 155 - DNA, 22 bp, Artificial sequence
  polynucleotide
ctttgtttataactctgagaag

SEQ ID NO: 156 - DNA, 22 bp, Artificial sequence
  polynucleotide
tcaaaatgcttttgatgcctga

SEQ ID NO: 157 - DNA, 1200 bp, Artificial sequence
  polynucleotide
atggacaaggcagagttgatccctgaaccacctaagaaaaagagaaaggtggagctcggaacagcagctaacttcaaccagtctggaaacattgcagactcttctttgtcttttactttcacaaattcttctaatggaccaaacttgattacaacacagacaaactcacaggctttgtctcagccaatcgcttcttctaatgtgcacgacaacttcatgaacaacgagattacagcttcaaagatcgatgacggtaacaattctaagcctctttctcctggatggactgaccagactgcatacaacgcattcggaatcacaacaggtatgttcaacacaactactatggatgatgtgtacaattacctttttgatgacgaggacacaccaccaaacccaaagaaagagggatcacttgagggtggatccggaggagacgtggtgatgacacagacaccattgtctttgcctgtgtccctaggagaccaggcatcaatctcatgcaggtcatctcagtctcttgtgcactctaatggtaacacttatttgaggtggtacttgcagaagccaggtcagtctccaaaggtgcttatctataaggtttctaacagattctcaggagtgccagataggttctcaggatcaggatctggaacagactttacattgaagatttcaagggttgaggcagaggaccttggagtgtacttctgctctcagtcaacacacgttccatggactttcggtggaggaacaaaacttgagattaaatctagcgctgacgacgctaagaaggacgctgctaagaaggatgacgctaaaaaggacgacgcaaagaaggacggtggtgtgaagcttgacgagactggaggtggtttggtgcagcctggaaggcctatgaaactttcatgcgtggcttctggattcacattctctgactactggatgaactgggttaggcagtcacctgagaagggtttggaatgggtggctcagatcaggaacaagccttacaactatgagacttactactctgattctgtgaaaggaaggttcactatctcaagggacgattcaaagtcttctgtttaccttcagatgaataacttacgcgtagaagacatgggtatctattactgtactggatcttactacggtatggactattggggacagggtacatcagtgacagtgtcatga

SEQ ID NO: 158 - DNA, 20 bp, Artificial sequence
  polynucleotide
tagggcgctggcaagtgtag

SEQ ID NO: 159 - DNA, 20 bp, Artificial sequence
  polynucleotide
cataacaccccttgtattac

SEQ ID NO: 160 - DNA, 1120 bp, Artificial sequence
  polynucleotide
caggtggcacttttcggggaaatgtgcgcggaacccctatttgtttatttttctaaatacattcaaatatgtatccgctcatgagacaataaccctgataaatgcttcaataatattgaaaaaggaagagtatgagtattcaacatttccgtgtcgcccttattcccttttttgcggcattttgccttcctgtttttgctcacccagaaacgctggtgaaagtaaaagatgctgaagatcagttgggtgcacgagtgggttacatcgaactggatctcaacagcggtaagatccttgagagttttcgccccgaagaacgttttccaatgatgagcacttttaaagttctgctatgtggcgcggtattatcccgtattgacgccgggcaagagcaactcggtcgccgcatacactattctcagaatgacttggttgagtactcaccagtcacagaaaagcatcttacggatggcatgacagtaagagaattatgcagtgctgccataaccatgagtgataacactgcggccaacttacttctgacaacgatcggaggaccgaaggagctaaccgcttttttgcacaacatgggggatcatgtaactcgccttgatcgttgggaaccggagctgaatgaagccataccaaacgacgagcgtgacaccacgatgcctgtagcaatggcaacaacgttgcgcaaactattaactggcgaactacttactctagcttcccggcaacaattaatagactggatggaggcggataaagttgcaggaccacttctgcgctcggcccttccggctggctggtttattgctgataaatctggagccggtgagcgtgggtctcgcggtatcattgcagcactggggccagatggtaagccctcccgtatcgtagttatctacacgacggggagtcaggcaactatggatgaacgaaatagacagatcgctgagataggtgcctcactgattaagcattggtaactgtcagaccaagtttactcatatatactttagattgatttaaaacttcatttttaatttaaaaggatctaggtgaagatcctttttgataatctcatgaacaataaaactgtctgcttacataaaca

SEQ ID NO: 161 - DNA, 21 bp, Artificial sequence
  polynucleotide
tatgagtattcaacatttccg

SEQ ID NO: 162 - DNA, 28 bp, Artificial sequence
  polynucleotide
  misc_feature (23)..(28): n is a, c, g, t or u
aataatattgaaaaaggaagagnnnnnn

SEQ ID NO: 163 - DNA, 28 bp, Artificial sequence
  polynucleotide
  misc_feature (1)..(6): n is a, c, g, t or u
nnnnnntgtcgcccttattccctttttt

SEQ ID NO: 164 - DNA, 28 bp, Artificial sequence
  polynucleotide
  misc_feature (1)..(6): n is a, c, g, t or u
nnnnnnctcttcctttttcaatattatt

SEQ ID NO: 165 - DNA, 28 bp, Artificial sequence
  polynucleotide
  misc_feature (23)..(28): n is a, c, g, t or u
aaaaaagggaataagggcgacannnnnn

SEQ ID NO: 166 - DNA, 24 bp, Artificial sequence
  polynucleotide
  misc_feature (23)..(24): n is a, c, g, t or u
caataatattgaaaaaggaagann

SEQ ID NO: 167 - DNA, 24 bp, Artificial sequence
  polynucleotide
  misc_feature (1)..(2): n is a, c, g, t or u
nntcgcccttattcccttttttgc

SEQ ID NO: 168 - DNA, 24 bp, Artificial sequence
  polynucleotide
  misc_feature (1)..(2): n is a, c, g, t or u
nntcttcctttttcaatattattg

SEQ ID NO: 169 - DNA, 24 bp, Artificial sequence
  polynucleotide
  misc_feature (23)..(24): n is a, c, g, t or u
gcaaaaaagggaataagggcgann

SEQ ID NO: 170 - DNA, 21 bp, Artificial sequence
  polynucleotide
agcattggtaactgtcagacc

SEQ ID NO: 171 - DNA, 28 bp, Artificial sequence
  polynucloeitde
  misc_feature (23)..(28): n is a, c, g, t or u
gagataggtgcctcactgattannnnnn

SEQ ID NO: 172 - DNA, 28 bp, Artificial sequence
  polynucleotide
  misc_feature (1)..(6): n is a, c, g, t or u
nnnnnnaagtttactcatatatacttta

SEQ ID NO: 173 - DNA, 28 bp, Artificial sequence
  polynucleotide
  misc_feature (1)..(6): n is a, c, g, t or u
nnnnnntaatcagtgaggcacctatctc

SEQ ID NO: 174 - DNA, 28 bp, Artificial sequence
  polynucleotide
  misc_feature (23)..(28): n is a, c, g, t or u
taaagtatatatgagtaaacttnnnnnn

SEQ ID NO: 175 - DNA, 24 bp, Artificial sequence
  polynucleotide
  misc_feature (23)..(24): n is a, c, g, t or u
tgagataggtgcctcactgattnn

SEQ ID NO: 176 - DNA, 24 bp, Artificial sequence
  polynucleotide
  misc_feature (1)..(2): n is a, c, g, t or u
nngtttactcatatatactttaga

SEQ ID NO: 177 - DNA, 24 bp, Artificial sequence
  polynucloeitde
  misc_feature (1)..(2): n is a, c, g, t or u
nnaatcagtgaggcacctatctca

SEQ ID NO: 178 - DNA, 24 bp, Artificial sequence
  polynucleotide
  misc_feature (23)..(24): n is a, c, g, t or u
tctaaagtatatatgagtaaacnn

SEQ ID NO: 179 - DNA, 1902 bp, Artificial sequence
  polynucleotide
gagtattctatagtgtcacctaaatagcttggcgtaatcatggtcatagctgtttcctgtgtgaaattgttatccgctcacaattccacacaacatacgagccggaagcataaagtgtaaagcctggggtgcctaatgagtgagctaactcacattaattgcgttgcgctcactgcccgctttccagtcgggaaacctgtcgtgccagctgcattaatgaatcggccaacgcgcggggagaggcggtttgcgtattgggcgctcttccgcttcctcgctcactgactcgctgcgctcggtcgttcggctgcggcgagcggtatcagctcactcaaaggcggtaatacggttatccacagaatcaggggataacgcaggaaagaacatgaattaattctcatgtttgacagcttatcatcgattagctttaatgcggtagtttatcacagttaaattgctaacgcagtcaggcaccgtgtatgaaatctaacaatgcgctcatcgtcatcctcggcaccgtcaccctggatgctgtaggcataggcttggttatgccggtactgccgggcctcttgcgggatatcgtccattccgacagcatcgccagtcactatggcgtgctgctagcgctatatgcgttgatgcaatttctatgcgcacccgttctcggagcactgtccgaccgctttggccgccgcccagtcctgctcgcttcgctacttggagccactatcgactacgcgatcatggcgaccacacccgtcctgtggattctctacgccggacgcatcgtggccggcatcaccggcgccacaggtgcggttgctggcgcctatatcgccgacatcaccgatggggaagatcgggctcgccacttcgggctcatgagcgcttgtttcggcgtgggtatggtggcaggccccgtggccgggggactgttgggcgccatctccttacatgcaccattccttgcggcggcggtgctcaacggcctcaacctactactgggctgcttcctaatgcaggagtcgcataagggagagcgccgaccgatgcccttgagagccttcaacccagtcagctccttccggtgggcgcggggcatgactatcgtcgccgcacttatgactgtcttctttatcatgcaactcgtaggacaggtgccggcagcgctctgggtcattttcggcgaggaccgctttcgctggagcgcgacgatgatcggcctgtcgcttgcggtattcggaatcttgcacgccctcgctcaagccttcgtcactggtcccgccaccaaacgtttcggcgagaagcaggccattatcgccggcatggcggccgacgcgctgggctacgtcttgctggcgttcgcgacgcgaggctggatggccttccccattatgattcttctcgcttccggcggcatcgggatgcccgcgttgcaggccatgctgtccaggcaggtagatgacgaccatcagggacagcttcaaggatcgctcgcggctcttaccagcctaacttcgatcactggaccgctgatcgtcacggcgatttatgccgcctcggcgagcacatggaacgggttggcatggattgtaggcgccgccctataccttgtctgcctccccgcgttgcgtcgcggtgcatggagccgggccacctcgacctgaatggaagccggcggcacctcgctaacggattcaccactccaagaattggagccaatcaattcttgcggagaactgtgaatgcgcaaaccaacccttgtatcggggaagaacagtatgtcgagctattttttgacttactggggatcaagcctgattgggagaaaataaaatattatattttactggatgaattgttttagtacctagatgtggcgcaacgatgccggcgaca

SEQ ID NO: 180 - DNA, 204 bp, Artificial sequence
  polynucleotide
ggactgtagaggttccgggtgacagccctccgacgggtgacagccctccgacgggtgacagccctccgaattctagaggatccgggtgacagccctccgacgggtgacagccctccgacgggtgacagccctccgaattcgagctcggtacccggggatctgtcgacctcgatcgagatcttcgcaagacccttcctctatata

SEQ ID NO: 181 - DNA, 1875 bp, Artificial sequence; identical to SEQ ID NO: 15
  polynucleotide

SEQ ID NO: 182 - DNA, 22 bp, Artificial sequence
  polynucleotide
atctcaagtctctaggactggt

SEQ ID NO: 183 - DNA, 22 bp, Artificial sequence
  polynucleotide
atctgtgagcaaaggcgaggag

SEQ ID NO: 184 - DNA, 68 bp, Artificial sequence
  polynucleotide
ccatgggatctcaagtctctaggactggtcttcaaaatctttctcactagtttctacgatcttggcca

SEQ ID NO: 185 - DNA, 62 bp, Artificial sequence
  polynucleotide
ccatgggatctcaagtctctaggactggtcaaaatctttctcactagtttctacgctggcca

SEQ ID NO: 186 - DNA, 56 bp, Artificial sequence
  polynucleotide
ccatgggatctcaagtctctaggactggtaatctttctcactagttacgctggcca

SEQ ID NO: 187 - DNA, 53 bp, Artificial sequence
  polynucleotide
ccatgggatctcaagtctctaggactggtaatctttcttgatcagtctggcca

SEQ ID NO: 188 - DNA, 52 bp, Artificial sequence
  polynucleotide
ccatgggatctcaagtctctaggactggtaatctttcttgatcagctggcca

SEQ ID NO: 189 - DNA, 51 bp, Artificial sequence
  polynucleotide
ccatgggatctcaagtctctaggactggtaatctttcttgatcactggcca

SEQ ID NO: 190 - DNA, 50 bp, Artificial sequence
  polynucleotide
ccatgggatctcaagtctctaggactggtctttctcactagttctggcca

SEQ ID NO: 191 - DNA, 44 bp, Artificial sequence
  polynucleotide
ccatgggatctcaagtctctaggactggtcttcactagtggcca

SEQ ID NO: 192 - DNA, 37 bp, Artificial sequence
  polynucleotide
aggaagttcatttcatttggrgaggacacgctgaacc

SEQ ID NO: 193 - DNA, 720 bp, Artificial sequence
  polynucleotide
atggtgagcaagggcgaggagctgttcaccggggtggtgcccatcctggtcgagctggacggcgacgtaaacggccacaagttcagcgtgtccggcgagggcgagggcgatgccacctacggcaagctgaccctgaagttcatctgcaccaccggcaagctgcccgtgccctggcccaccctcgtgaccaccctgacctacggcgtgcagtgcttcagccgctaccccgaccacatgaagcagcacgacttcttcaagtccgccatgcccgaaggctacgtccaggagcgcaccatcttcttcaaggacgacggcaactacaagacccgcgccgaggtgaagttcgagggcgacaccctggtgaaccgcatcgagctgaagggcatcgacttcaaggaggacggcaacatcctggggcacaagctggagtacaactacaacagccacaacgtctatatcatggccgacaagcagaagaacggcatcaaggtgaacttcaagatccgccacaacatcgaggacggcagcgtgcagctcgccgaccactaccagcagaacacccccatcggcgacggccccgtgctgctgcccgacaaccactacctgagcacccagtccgccctgagcaaagaccccaacgagaagcgcgatcacatggtcctgctggagttcgtgaccgccgccgggatcactctcggcatggacgagctgtacaagtaa

SEQ ID NO: 194 - DNA, 1809 bp, Artificial sequence
  polynucleotide
atgttacgtcctgtagaaaccccaacccgtgaaatcaaaaaactcgacggcctgtgggcattcagtctggatcgcgaaaactgtggaattgatcagcgttggtgggaaagcgcgttacaagaaagccgggcaattgctgtgccaggcagttttaacgatcagttcgccgatgcagatattcgtaattatgcgggcaacgtctggtatcagcgcgaagtctttataccgaaaggttgggcaggccagcgtatcgtgctgcgtttcgatgcggtcactcattacggcaaagtgtgggtcaataatcaggaagtgatggagcatcagggcggctatacgccatttgaagccgatgtcacgccgtatgttattgccgggaaaagtgtacgtatcaccgtttgtgtgaacaacgaactgaactggcagactatcccgccgggaatggtgattaccgacgaaaacggcaagaaaaagcagtcttacttccatgatttctttaactatgccggaatccatcgcagcgtaatgctctacaccacgccgaacacctgggtggacgatatcaccgtggtgacgcatgtcgcgcaagactgtaaccacgcgtctgttgactggcaggtggtggccaatggtgatgtcagcgttgaactgcgtgatgcggatcaacaggtggttgcaactggacaaggcactagcgggactttgcaagtggtgaatccgcacctctggcaaccgggtgaaggttatctctatgaactgtgcgtcacagccaaaagccagacagagtgtgatatctacccgcttcgcgtcggcatccggtcagtggcagtgaagggccaacagttcctgattaaccacaaaccgttctactttactggctttggtcgtcatgaagatgcggacttacgtggcaaaggattcgataacgtgctgatggtgcacgaccacgcattaatggactggattggggccaactcctaccgtacctcgcattacccttacgctgaagagatgctcgactgggcagatgaacatggcatcgtggtgattgatgaaactgctgctgtcggctttaacctctctttaggcattggtttcgaagcgggcaacaagccgaaagaactgtacagcgaagaggcagtcaacggggaaactcagcaagcgcacttacaggcgattaaagagctgatagcgcgtgacaaaaaccacccaagcgtggtgatgtggagtattgccaacgaaccggatacccgtccgcaagtgcacgggaatatttcgccactggcggaagcaacgcgtaaactcgacccgacgcgtccgatcacctgcgtcaatgtaatgttctgcgacgctcacaccgataccatcagcgatctctttgatgtgctgtgcctgaaccgttattacggatggtatgtccaaagcggcgatttggaaacggcagagaaggtactggaaaaagaacttctggcctggcaggagaaactgcatcagccgattatcatcaccgaatacggcgtggatacgttagccgggctgcactcaatgtacaccgacatgtggagtgaagagtatcagtgtgcatggctggatatgtatcaccgcgtctttgatcgcgtcagcgccgtcgtcggtgaacaggtatggaatttcgccgattttgcgacctcgcaaggcatattgcgcgttggcggtaacaagaaagggatcttcactcgcgaccgcaaaccgaagtcggcggcttttctgctgcaaaaacgctggactggcatgaacttcggtgaaaaaccgcagcagggaggcaaacaatga

SEQ ID NO: 195 - DNA, 211 bp, Artificial sequence
  polynucleotide
gtccgcaaaaatcaccagtctctctctacaaatctatctctctctatttttctccagaataatgtgtgagtagttcccagataagggaattagggttcttatagggtttcgctcatgtgttgagcatataagaaacccttagtatgtatttgtatttgtaaaatacttctatcaataaaatttctaattcctaaaaccaaaatccagtgac

SEQ ID NO: 196 - DNA, 24 bp, Artificial sequence
  polynucleotide
  misc_feature (19)..(24): n is a, c, g, t or u
cgggtgacagccctccgannnnnn

SEQ ID NO: 197 - DNA, 24 bp, Artificial sequence
  polynucleotide
  misc_feature (1)..(6): n is a, c, g, t or u
nnnnnntcggagggctgtcacccg

SEQ ID NO: 198 - DNA, 152 bp, Artificial sequence
  polynucleotide
tcttcgctattacgccagctggcgaaagggggatgtgctgcaaggcgattaagttgggtaacgccagggttttcccagtcacgacgttgtaaaacgacggccagtgccacccataatacccataatagctgtttgccaaccggttctatata

SEQ ID NO: 199 - DNA, 37 bp, Artificial sequence; identical to SEQ ID NO: 192
  polynucleotide

SEQ ID NO: 200 - DNA, 720 bp, Artificial sequence; identical to SEQ ID NO: 193
  polynucleotide

SEQ ID NO: 201 - DNA, 1809 bp, Artificial sequence; identical to SEQ ID NO: 194
  polynucleotide

SEQ ID NO: 202 - DNA, 211 bp, Artificial sequence; identical to SEQ ID NO: 195
  polynucloeitde

SEQ ID NO: 203 - DNA, 28 bp, Artificial sequence
  polynucleotide
  misc_feature (23)..(28): n is a, c, g, t or u
gccagggttttcccagtcacgannnnnn

SEQ ID NO: 204 - DNA, 28 bp, Artificial sequence
  polynucleotide
  misc_feature (1)..(6): n is a, c, g, t or u
nnnnnntcgtgactgggaaaaccctggc

SEQ ID NO: 205 - protein, 238 aa, Artificial sequence
  polypeptide
MHSRSALLYRFLRPASRCFSSSSVKSELEEKKSELRHKLKYVPHEYIELIEIARNSTQDRILEMKVMEFFMKVYGYRGKHLGGSRKPDGAIYTVGSPIDYGVIVDTKAYSGGYNLPIGQADEMQRYVEENQTRNKHINPNEWWKVYPSSVTEFKFLFVSGHFKGNYKAQLTRLNHITNCNGAVLSVEELLIGGEMIKAGTLTLEEVRRKFNNGEINFGSGGSGPRPRGTRGKGRRIRR

SEQ ID NO: 206 - DNA, 717 bp, Artificial sequence
  polynucleotide
atgcattctagatctgctcttctttatagatttcttagaccagcttctagatgtttttcttcttcttctgttaagtctgaacttgaagaaaagaagtctgaacttagacataagcttaagtatgttccacatgaatatattgaacttattgaaattgctagaaattctactcaagatagaattcttgaaatgaaggttatggaattttttatgaaggtttatggatatagaggaaagcatcttggaggatctagaaagccagatggagctatttatactgttggatctccaattgattatggagttattgttgatactaaggcttattctggaggatataatcttccaattggacaagctgatgaaatgcaaagatatgttgaagaaaatcaaactagaaataagcatattaatccaaatgaatggtggaaggtttatccatcttctgttactgaatttaagtttctttttgtttctggacattttaagggaaattataaggctcaacttactagacttaatcatattactaattgtaatggagctgttctttctgttgaagaacttcttattggaggagaaatgattaaggctggaactcttactcttgaagaagttagaagaaagtttaataatggagaaattaattttggatctggaggatctggaccaagaccaagaggaactagaggaaagggaagaagaattagaagataa

SEQ ID NO: 207 - DNA, 43 bp, Artificial sequence
  polynucleotide
  misc_feature (21)..(21): n is a, c, g, t or u
uucaccucuaaccgggugagnuccaagggcgaggagcuguuca

SEQ ID NO: 208 - DNA, 43 bp, Artificial sequence
  polynucleotide
  misc_feature (23)..(23): n is a, c, g, t or u
accauuuacgaacgauagccaunuucaccucuaaccgggugag

SEQ ID NO: 209 - DNA, 43 bp, Artificial sequence
  polynucleotide
  misc_feature (21)..(21): n is a, c, g, t or u
uucaccucuaaccgggugagnauggcuaucguucguaaauggu

SEQ ID NO: 210 - DNA, 43 bp, Artificial sequence
  polynucleotide
  misc_feature (23)..(23): n is a, c, g, t or u
ugaacagcuccucgcccuugganuucaccucuaaccgggugag

SEQ ID NO: 211 - DNA, 24 bp, Artificial sequence
  polynucleoitde
  misc_feature (1)..(2): n is a, c, g, t or u
nntgtccaagggcgaggagctgtt

SEQ ID NO: 212 - DNA, 24 bp, Artificial sequence
  polynucleotide
  misc_feature (23)..(24): n is a, c, g, t or u
catttacgaacgatagccatggnn

SEQ ID NO: 213 - DNA, 24 bp, Artificial sequence
  polynucleotide
  misc_feature (1)..(2): n is a, c, g, t or u
nnccatggctatcgttcgtaaatg

SEQ ID NO: 214 - DNA, 24 bp, Artificial sequence
  polynucleotide
  misc_feature (23)..(24): n is a, c, g, t or u
aacagctcctcgcccttggacann

SEQ ID NO: 215 - protein, 6 aa, Artificial sequence
  peptide
ACTAGT

SEQ ID NO: 216 - protein, 6 aa, Artificial sequence
  peptide
TGATCA

SEQ ID NO: 217 - DNA, 28 bp, Artificial sequence
  polynucleotide
  misc_feature (23)..(28): n is a, c, g, t or u
ataccagcaccagcaattacaannnnnn